European Patent Application EP 4 285 935 A1, published December 6, 2023. Title: Novel Anti-Nectin-4 Antibody Camptothecin derivative Conjugates. Applicant: Emergence Therapeutics AG, et al. The sequence listing filed with the application follows.

SEQUENCE LISTING (111 sequences)

SEQ ID NO: 1 - protein, 8 aa, artificial sequence
  CDR1 VH_15A7.5 IMGT
GFTFSNYG

SEQ ID NO: 2 - protein, 8 aa, artificial sequence
  CDR2 VH_15A7.5 IMGT
ISNLAYGI

SEQ ID NO: 3 - protein, 12 aa, artificial sequence
  CDR3 VH_15A7.5 IMGT
ARGARATGWFAY

SEQ ID NO: 4 - protein, 6 aa, artificial sequence
  CDR1 VK_15A7.5 IMGT
QNVDTH

SEQ ID NO: 5 - protein, 3 aa, artificial sequence
  CDR2 VK_15A7.5 IMGT
SAS

SEQ ID NO: 6 - protein, 9 aa, artificial sequence
  CDR3 VK_15A7.5 IMGT
QQYNSYPLT

SEQ ID NO: 7 - protein, 5 aa, artificial sequence
  CDR1 VH_15A7.5 Kabat
NYGMA

SEQ ID NO: 8 - protein, 17 aa, artificial sequence
  CDR2 VH_15A7.5 Kabat
FISNLAYGINYADTVTG

SEQ ID NO: 9 - protein, 10 aa, artificial sequence
  CDR3 VH_15A7.5 Kabat
GARATGWFAY

SEQ ID NO: 10 - protein, 11 aa, artificial sequence
  CDR1 VK_15A7.5 Kabat
KASQNVDTHVA

SEQ ID NO: 11 - protein, 7 aa, artificial sequence
  CDR2 VK_15A7.5 Kabat
SASYRYS

SEQ ID NO: 12 - protein, 9 aa, artificial sequence
  CDR3 VK_15A7.5 Kabat
QQYNSYPLT

SEQ ID NO: 13 - protein, 119 aa, artificial sequence
  VH_15A7.5
EVKLVESGGGLVQPGGSRKLSCAASGFTFSNYGMAWVRQAPGKGPEWVAFISNLAYGINYADTVTGRFTISRENAKNTLYLEMRSLRSEDTAMYYCARGARATGWFAYWGQGTLVTVSA

SEQ ID NO: 14 - protein, 107 aa, artificial sequence
  VK_15A7.5
DIVMTQSQKFMSTSIGDRVSVTCKASQNVDTHVAWYQEKPGQSPKALIYSASYRYSGVPDRFTGSGSGTDFTLTISNVQSEDLADYFCQQYNSYPLTFGGGTKLEIK

SEQ ID NO: 15 - protein, 9 aa, artificial sequence
  CDR1 H0_15A7.5  IMGT
GFTFSNYGM

SEQ ID NO: 16 - protein, 8 aa, artificial sequence
  CDR2 H0_15A7.5  IMGT
ISNLAYGI

SEQ ID NO: 17 - protein, 12 aa, artificial sequence
  CDR3 H0_15A7.5  IMGT
ARGARATGWFAY

SEQ ID NO: 18 - protein, 6 aa, artificial sequence
  CDR1 L0_15A7.5 IMGT
QNVDTH

SEQ ID NO: 19 - protein, 3 aa, artificial sequence
  CDR2 L0_15A7.5 IMGT
SAS

SEQ ID NO: 20 - protein, 9 aa, artificial sequence
  CDR3 L0_15A7.5 IMGT
QQYNSYPLT

SEQ ID NO: 21 - protein, 5 aa, artificial sequence
  CDR1 H0_15A7.5  Kabat
NYGMN

SEQ ID NO: 22 - protein, 17 aa, artificial sequence
  CDR2 H0_15A7.5  Kabat
FISNLAYGINYADSVKG

SEQ ID NO: 23 - protein, 10 aa, artificial sequence
  CDR3 H0_15A7.5  Kabat
GARATGWFAY

SEQ ID NO: 24 - protein, 11 aa, artificial sequence
  CDR1 L0_15A7.5 Kabat
RASQNVDTHVA

SEQ ID NO: 25 - protein, 7 aa, artificial sequence
  CDR2 L0_15A7.5 Kabat
SASYLQS

SEQ ID NO: 26 - protein, 9 aa, artificial sequence
  CDR3 L0_15A7.5 Kabat
QQYNSYPLT

SEQ ID NO: 27 - protein, 119 aa, artificial sequence
  H0_15A7.5
EVQLVESGGGLVQPGGSLRLSCAASGFTFSNYGMNWVRQAPGKGLEWVSFISNLAYGINYADSVKGRFTISRDNAKNSLYLQMNSLRAEDTAVYYCARGARATGWFAYWGQGTLVTVSS

SEQ ID NO: 28 - protein, 107 aa, artificial sequence
  L0_15A7.5
DIQMTQSPSSLSASVGDRVTITCRASQNVDTHVAWFQQKPGKAPKSLIYSASYLQSGVPSRFSGSGSGTDFTLTISSLQPEDFATYYCQQYNSYPLTFGGGTKVEIK

SEQ ID NO: 29 - protein, 8 aa, artificial sequence
  CDR1 H1_15A7.5 IMGT
GFTFSNYG

SEQ ID NO: 30 - protein, 8 aa, artificial sequence
  CDR2 H1_15A7.5 IMGT
ISNLAYGI

SEQ ID NO: 31 - protein, 12 aa, artificial sequence
  CDR3 H1_15A7.5 IMGT
ARGARATGWFAY

SEQ ID NO: 32 - protein, 6 aa, artificial sequence
  CDR1 L1_15A7.5 IMGT
QNVDTH

SEQ ID NO: 33 - protein, 3 aa, artificial sequence
  CDR2 L1_15A7.5 IMGT
SAS

SEQ ID NO: 34 - protein, 9 aa, artificial sequence
  CDR3 L1_15A7.5 IMGT
QQYNSYPLT

SEQ ID NO: 35 - protein, 5 aa, artificial sequence
  CDR1 H1_15A7.5 Kabat
NYGMA

SEQ ID NO: 36 - protein, 17 aa, artificial sequence
  CDR2 H1_15A7.5 Kabat
FISNLAYGINYADTVTG

SEQ ID NO: 37 - protein, 10 aa, artificial sequence
  CDR3 H1_15A7.5 Kabat
GARATGWFAY

SEQ ID NO: 38 - protein, 11 aa, artificial sequence
  CDR1 L1_15A7.5 Kabat
KASQNVDTHVA

SEQ ID NO: 39 - protein, 7 aa, artificial sequence
  CDR2 L1_15A7.5 Kabat
SASYRYS

SEQ ID NO: 40 - protein, 9 aa, artificial sequence
  CDR3 L1_15A7.5 Kabat
QQYNSYPLT

SEQ ID NO: 41 - protein, 119 aa, artificial sequence
  H1_15A7.5
EVQLVESGGGLVQPGGSLRLSCAASGFTFSNYGMAWVRQAPGKGLEWVSFISNLAYGINYADTVTGRFTISRDNAKNSLYLQMNSLRAEDTAVYYCARGARATGWFAYWGQGTLVTVSS

SEQ ID NO: 42 - protein, 108 aa, artificial sequence
  L1_15A7.5
DIQMTQSPSSLSASVGDRVTITCCKASQNVDTHVAWFQQKPGKAPKSLIYSASYRYSGVPSRFSGSGSGTDFTLTISSLQPEDFATYYCQQYNSYPLTFGGGTKVEIK

SEQ ID NO: 43 - protein, 8 aa, artificial sequence
  CDR1 H2_15A7.5 IMGT
GFTFSNYG

SEQ ID NO: 44 - protein, 8 aa, artificial sequence
  CDR2 H2_15A7.5 IMGT
ISNLAYGI

SEQ ID NO: 45 - protein, 12 aa, artificial sequence
  CDR3 H2_15A7.5 IMGT
ARGARATGWFAY

SEQ ID NO: 46 - protein, 6 aa, artificial sequence
  CDR1 L2_15A7.5 IMGT
QNVDTH

SEQ ID NO: 47 - protein, 3 aa, artificial sequence
  CDR2 L2_15A7.5 IMGT
SAS

SEQ ID NO: 48 - protein, 9 aa, artificial sequence
  CDR3 L2_15A7.5 IMGT
QQYNSYPLT

SEQ ID NO: 49 - protein, 5 aa, artificial sequence
  CDR1 H2_15A7.5 Kabat
NYGMA

SEQ ID NO: 50 - protein, 17 aa, artificial sequence
  CDR2 H2_15A7.5 Kabat
FISNLAYGINYADTVTG

SEQ ID NO: 51 - protein, 10 aa, artificial sequence
  CDR3 H2_15A7.5 Kabat
GARATGWFAY

SEQ ID NO: 52 - protein, 11 aa, artificial sequence
  CDR1 L2_15A7.5 Kabat
KASQNVDTHVA

SEQ ID NO: 53 - protein, 7 aa, artificial sequence
  CDR2 L2_15A7.5 Kabat
SASYRYS

SEQ ID NO: 54 - protein, 9 aa, artificial sequence
  CDR3 L2_15A7.5 Kabat
QQYNSYPLT

SEQ ID NO: 55 - protein, 119 aa, artificial sequence
  H2_15A7.5
EVQLVESGGGLVQPGGSLRLSCAASGFTFSNYGMAWVRQAPGKGLEWVAFISNLAYGINYADTVTGRFTISRDNAKNSLYLQMNSLRAEDTAVYYCARGARATGWFAYWGQGTLVTVSS

SEQ ID NO: 56 - protein, 107 aa, artificial sequence
  L2_15A7.5
DIQMTQSPSSLSASVGDRVTITCKASQNVDTHVAWYQQKPGKAPKALIYSASYRYSGVPSRFSGSGSGTDFTLTISSLQPEDFATYYCQQYNSYPLTFGGGTKVEIK

SEQ ID NO: 57 - protein, 8 aa, artificial sequence
  CDR1 H3_15A7.5 IMGT
GFTFSNYG

SEQ ID NO: 58 - protein, 8 aa, artificial sequence
  CDR2 H3_15A7.5 IMGT
ISNLAYGI

SEQ ID NO: 59 - protein, 12 aa, artificial sequence
  CDR3 H3_15A7.5 IMGT
ARGARATGWFAY

SEQ ID NO: 60 - protein, 6 aa, artificial sequence
  CDR1 L3_15A7.5 IMGT
QNVDTH

SEQ ID NO: 61 - protein, 3 aa, artificial sequence
  CDR2 L3_15A7.5 IMGT
SAS

SEQ ID NO: 62 - protein, 9 aa, artificial sequence
  CDR3 L3_15A7.5 IMGT
QQYNSYPLT

SEQ ID NO: 63 - protein, 5 aa, artificial sequence
  CDR1 H3_15A7.5 Kabat
NYGMA

SEQ ID NO: 64 - protein, 17 aa, artificial sequence
  CDR2 H3_15A7.5 Kabat
FISNLAYGINYADTVTG

SEQ ID NO: 65 - protein, 10 aa, artificial sequence
  CDR3 H3_15A7.5 Kabat
GARATGWFAY

SEQ ID NO: 66 - protein, 11 aa, artificial sequence
  CDR1 L3_15A7.5 Kabat
KASQNVDTHVA

SEQ ID NO: 67 - protein, 7 aa, artificial sequence
  CDR2 L3_15A7.5 Kabat
SASYRYS

SEQ ID NO: 68 - protein, 9 aa, artificial sequence
  CDR3 L3_15A7.5 Kabat
QQYNSYPLT

SEQ ID NO: 69 - protein, 119 aa, artificial sequence
  H3_15A7.5
EVQLVESGGGLVQPGGSLRLSCAASGFTFSNYGMAWVRQAPGKGPEWVAFISNLAYGINYADTVTGRFTISRDNAKNSLYLQMNSLRAEDTAVYYCARGARATGWFAYWGQGTLVTVSS

SEQ ID NO: 70 - protein, 108 aa, artificial sequence
  L3_15A7.5
DIQMTQSPSSLSASVGDRVTITCKASQNVDTHVAWYYQQKPGKSPKALIYSASYRYSGVPSRFSGSGSGTDFTLTISSLQPEDFATYYCQQYNSYPLTFGGGTKVEIK

SEQ ID NO: 71 - protein, 107 aa, artificial sequence
  L3_15A7.5_mod
DIQMTQSPSSLSASVGDRVTITCKASQNVDTHVAWYYQQKPGKSPKALIYSASYRYSGVPSRFSGSGSGTDFTLTISSLQPEDFATYCQQYNSYPLTFGGGTKVEIK

SEQ ID NO: 72 - protein, 8 aa, artificial sequence
  CDR1 VH_HA22
GFTFSSYN

SEQ ID NO: 73 - protein, 8 aa, artificial sequence
  CDR2 VH_HA22
ISSSSSTI

SEQ ID NO: 74 - protein, 10 aa, artificial sequence
  CDR3 VH_HA22
ARAYYYGMDV

SEQ ID NO: 75 - protein, 6 aa, artificial sequence
  CDR1 VK_HA22
QGISGW

SEQ ID NO: 76 - protein, 3 aa, artificial sequence
  CDR2 VK_HA22
AAS

SEQ ID NO: 77 - protein, 9 aa, artificial sequence
  CDR3 VK_HA22
QQANSFPPT

SEQ ID NO: 78 - protein, 117 aa, artificial sequence
  VH_HA22
EVQLVESGGGLVQPGGSLRLSCAASGFTFSSYNMNWVRQAPGKGLEWVSYISSSSSTIYYADSVKGRFTISRDNAKNSLSLQMNSLRDEDTAVYYCARAYYYGMDVWGQGTTVTVSS

SEQ ID NO: 79 - protein, 107 aa, artificial sequence
  VK_HA22
DIQMTQSPSSVSASVGDRVTITCRASQGISGWLAWYQQKPGKAPKFLIYAASTLQSGVPSRFSGSGSGTDFTLTISSLQPEDFATYYCQQANSFPPTFGGGTKVEIK

SEQ ID NO: 80 - protein, 8 aa, artificial sequence
  CDR1 VH_5A12.2
GFTFNSMY

SEQ ID NO: 81 - protein, 8 aa, artificial sequence
  CDR2 VH_5A12.2
IYAGTGGT

SEQ ID NO: 82 - protein, 13 aa, artificial sequence
  CDR3 VH_5A12.2
AIRSGFVPMDYWG

SEQ ID NO: 83 - protein, 118 aa, artificial sequence
  VH_5A12.2
QIQLQQSGAELVKPGASVTLSCKTSGFTFNSMYISWLKQKPGQSLEWIAWIYAGTGGTRFNQKFTGKVQLTVDTSSSTAYMQFSSLTTDDSAIYYCAIRSGFVPMDYWGQGTSVTVSS

SEQ ID NO: 84 - protein, 6 aa, artificial sequence
  CDR1 VK_5A12.2
QSVSND

SEQ ID NO: 85 - protein, 3 aa, artificial sequence
  CDR2 VK_5A12.2
YAS

SEQ ID NO: 86 - protein, 6 aa, artificial sequence
  CDR3 VK_5A12.2
QQDYSS

SEQ ID NO: 87 - protein, 107 aa, artificial sequence
  VK_5A12.2
SIVMTQTPKFLLVSAGDRVTITCKASQSVSNDVAWYQQKPGQSPKLLIYYASNRYTGVPDRFTGSGYGTDFTFTISTVQAEDLAVYFCQQDYSSPWTFGGGTKLEIK

SEQ ID NO: 88 - protein, 8 aa, artificial sequence
  CDR1 VH_9A2.7
GYNFTTFW

SEQ ID NO: 89 - protein, 8 aa, artificial sequence
  CDR2 VH_9A2.7
IYPSDSYA

SEQ ID NO: 90 - protein, 13 aa, artificial sequence
  CDR3 VH_9A2.7
TRPSYFGRNSFAY

SEQ ID NO: 91 - protein, 120 aa, artificial sequence
  VH_9A2.7
QVQLQQPGAELVRPGASVKLSCKASGYNFTTFWINWVKQRPGQGLEWIGNIYPSDSYANYNQKFKDKATLTVDKSSTTAYMQLSSPTSEDSAVYYCTRPSYFGRNSFAYWGQGTLVTVSA

SEQ ID NO: 92 - protein, 12 aa, artificial sequence
  CDR1 VK_9A2.7
QSLLYSVNHKNY

SEQ ID NO: 93 - protein, 3 aa, artificial sequence
  CDR2 VK_9A2.7
WAS

SEQ ID NO: 94 - protein, 9 aa, artificial sequence
  CDR3 VK_9A2.7
HQYYTYPLT

SEQ ID NO: 95 - protein, 113 aa, artificial sequence
  VK_9A2.7
DIVMTQSPSSLVVSVGEKVTMSCKSSQSLLYSVNHKNYLAWYQQKPGQSPKLLIYWASTRESGVPDRFTGSGSGTDFSLTISSVKAEDLAVYYCHQYYTYPLTFGAGTKLELK

SEQ ID NO: 96 - protein, 8 aa, artificial sequence
  CDR1 VH_3A1.4
GDSITSGY

SEQ ID NO: 97 - protein, 7 aa, artificial sequence
  CDR2 VH_3A1.4
ISNSGIT

SEQ ID NO: 98 - protein, 15 aa, artificial sequence
  CDR3 VH_3A1.4
TRFGSTMILYYTMDY

SEQ ID NO: 99 - protein, 121 aa, artificial sequence
  VH_3A1.4
DVQLQESGPSLVKPSQTLSLTCSVTGDSITSGYWNWIRKFPGNKLEYMGYISNSGITYYNPSLKSRISITRDTSKNQYFLQLNSVTAEDTATYYCTRFGSTMILYYTMDYWGQGTSVTVSS

SEQ ID NO: 100 - protein, 6 aa, artificial sequence
  CDR1 VK_3A1.4
QSISDY

SEQ ID NO: 101 - protein, 3 aa, artificial sequence
  CDR2 VK_3A1.4
YAS

SEQ ID NO: 102 - protein, 9 aa, artificial sequence
  CDR3 VK_3A1.4
QNGHSFPLT

SEQ ID NO: 103 - protein, 107 aa, artificial sequence
  VK_3A1.4
DIVMTQSPVTLSVTPGDRVSLSCRASQSISDYLHWYQQKSQESPRLLIKYASKSISGIPSRFSGSGSGSNFTLSINSVEPEDVGVYYCQNGHSFPLTFGAGTKLELK

SEQ ID NO: 104 - protein, 8 aa, artificial sequence
  CDR1 VH_8F06
GYTFTSYV

SEQ ID NO: 105 - protein, 8 aa, artificial sequence
  CDR2 VH_8F06
INPYNDGT

SEQ ID NO: 106 - protein, 6 aa, artificial sequence
  CDR3 VH_8F06
VTLFAY

SEQ ID NO: 107 - protein, 113 aa, artificial sequence
  VH_8F06
EVQLQQSGPELVKPGASVKMSCKASGYTFTSYVMHWVKQKPGQGLEWIGYINPYNDGTKYNEKFKGKATLTSDKSSSTAYMELSSLTSEDSAVYYCVTLFAYWGQGTLVTVSA

SEQ ID NO: 108 - protein, 5 aa, artificial sequence
  CDR1 VK_8F06
SSISY

SEQ ID NO: 109 - protein, 3 aa, artificial sequence
  CDR2 VK_8F06
DTS

SEQ ID NO: 110 - protein, 9 aa, artificial sequence
  CDR3 VK_8F06
HQRSSYPFT

SEQ ID NO: 111 - protein, 106 aa, artificial sequence
  VK_8F06
QIVLTQSPAIMSASPGEKVTMTCSASSSISYMHWYQQKPGTSPKRWIYDTSKLASGVPARFSGSGSGTSYSLTISSMEAEDAATYYCHQRSSYPFTFGSGTKLEIK